European Patent Application EP 4 170 038 A1, published April 26, 2023. Title: Pichia ciferrii mutant strains Having Enhanced Spingoid Base and Sphingolipid Production And Preparation Method of the same. Applicant: Doosan Solus co., Ltd. Korea Research Institute of Bioscience and Biotechnology. The sequence listing filed with the application follows.

SEQUENCE LISTING (29 sequences)

SEQ ID NO: 1 - DNA, 1647 bp, Pichia ciferrii
  gene (1)..(1647): GAPDH, glyceraldehyde 3-phosphate dehydrogenase (GAPDH) gene
aagcaattaaacaacataccaacaaaacaattatacccagtgatacctacatacaattaacccatagtaaactaatacctcacaacattaataaagcatctgatcttaatgtactactaatcctaaactcatgataattactgctgttgtaatgtttgtcatcactttgatcatcacgagcatcaccggaccgttaattaccaacaatctcaattgtagaacacagtgttaaacagggataaaacaacaattaattatgataaaaggttcaaacaagtaccaatagatagataattattacctctataatatatcatttaattgaattaatatcaatagttgttattcaattatccctactttcctggttaaagttacaccatcagatggttcaccaccaatgttgttcaaaccatttccactcaactgacgtttcaacaacatcacctgaaaaaaaaattcatcacacattgggagaaattgggagaattgtatataaggagttgaaatcgctaattattttatacttcttcattatacttctattctacatcagtattttataatacaaaaacaaacaaataaaacaaataattaacaatggctatcacagttggtattaacggtttcggtcgtattggtcgtttagtcctaagaattgctctttcaagaaaagatattcaaattgttgcaattaatgatccattcattgcaccagaatatgcttcatatatgtttaaatatgattctactcatggtcgttatgcaggtgaagtttctcatgaaggtgataacattgttattgatggtaaaaaaatcagagtttatcaagaacgtgatccagttaacatcccatggggtaaagatggtgttgattatgttattgattcaactggtgtttttaaagaattagattctgctcaaaaacatattgatgccggtgctaaaaaagttgttattactgctccatcatcaactgctccaatgtttgttgttggtgttaatgaagataaatatactccagatttaaacattatttcaaatgcttcatgtacaacaaattgtttagctccattagctaaaattattaacaacaaatttggtattgaagaaggtttaatgactactgttcattcaattactgctactcaaaaaactgttgatggtccatctcataaagattggagaggtggtcgtactgcttcaggtaatattattccatcatcaactggtgctgctaaagctgttggtaaagttattccagaattagctggtaaattaactggtatgtctttaagagttccaactgttgatgtttcagttgttgatttaactgttaaattattaaaagatgccacttatgatgaaattaaagctgctgttaaagaagctgctgaaggtccattaaaaggtgttgttggttatactgaagatcaagttgtttcttcagatttcttgactgataacagatcatcaattttcgatgctgaagctggtatttggttatcaccaagatttgttaaattaattgcttggtatgataatgaatatggttactctaccagagttgttgatttattagaatacgttgcttcaaaaactaagaaacgaaagctaatgaaaagcaatagctttgaattagtttga

SEQ ID NO: 2 - DNA, 576 bp, Artificial Sequence
  nat1
atgggtactactttagatgatactgcttatagatatagaacttcagttccaggtgatgctgaagctattgaagctttagatggttcatttactactgatactgtttttagagttactgctactggtgatggttttactttaagagaagttccagttgatccaccattaactaaagtttttccagatgatgaatcagatgacgagtctgatgacggtgaagatggtgatccagattcaagaacttttgttgcttatggtgatgacggagacttagctggttttgttgttgtttcatattcaggttggaatagaagattaactgttgaagatattgaagttgctccagaacatagaggtcatggtgttggtagagctttaatgggtttagctactgaatttgctagagaacgtggtgctggtcatttatggttagaagttactaatgttaatgctccagctattcatgcttatagaagaatgggtttcacattatgtggtttagatactgctttatatgatggtactgcttcagatggtgaacaagctttatatatgtcaatgccatgtccataataa

SEQ ID NO: 3 - DNA, 1591 bp, Pichia ciferrii
  gene (1)..(1591): URA3, orotidine-5'-phosphate decarboxylase (URA3) gene
gattgatttgatatagatttgagctttgtagttctgatctattaggtacaaaaggtctttcaatggcaaaagtgtacttttttgatttttcaatgaagtcgaaaaggttcaaattttttttgtcaacaaaacatcataaatacccggatttggcaagtatcccgatatggtcatactcaggaaccaattgatatcattatttatttaggcattaaagtgtgaataattctttgtgatatcagtactttattatatcaagcttgaaagggatactaggtgatccattgatcgaatctgctcttcttttcaaccttctcaaagaaacaaaattgttgcttaattttggctgttgtagaacttgtacgggacacgcttctatgaacaaatttgtccgatgagttggataaatattactttcctttgattgatagcacatcatcaatagattgcaaatataatccaaaatggtcaccacattatcttacactcaaaggcagaagctcacccttctccattggcaaagcgtttattcaatgtcatggaatcaaaaaagtcaaacttgtgtgcttcaattgatgttagaactacaaaagaatttttacaattagttgacacattaggtccatatatctgtcttgtcaaaactcatatcgatattattgatgatttctcatttgaaggtactatcaaaccattgagagaattagcacaaaagcacaattttttaatctttgaagatcgtaaatttgctgatatagggaacacagtcaaagcacaatatgcaggtggtgctttcaaaattgcaacttggtctgatatcacaaatgctcatggtgttactggtgctggtatcgttagtgggttgaaagaggctgctaaagaagcttcagatgaaccaagaggtttgttgatgttggctgaattgagttcaaaaggttcattagccaaaggtgaatatactaaacaaactgttgatatcgctaaaactgataaagattttgttattggatttattgctcaaaatgatatgggtggtagagatgaaggctttgattggttaatcatgacccaggtgttggtcttgatgataaaggtgatgccttaggtcaacaatatagatctgttgatactgtcgtttcaactggtagtgatatcattattgtcggtagaggtttattcggtaaaggaagagatccaaatgctgaaggtgaacgttacagagctgctggttggaatgcttatttgaaaagaactggtcaaatatagaatgtagtttaaatataaaatattagactaaataattaatgggtgctagtttgtaactagttcaacgactataattaactgacattaaaagtagctgactctaagtgtattcaatgtcattcatactgctaatcaaataaatcaaaatatacattgaagtttgtatcattaattagaagatgttataatgtcgatgactaagcaagtaaattaaaaccgaaatccatctgtatgtaaaaatacttcaaagtcttaacagcatagatagaagcttatcaatcaactatcatcaagccagtagatgccattcaaaagtgacaaatgt

SEQ ID NO: 4 - DNA, 2983 bp, Artificial Sequence
  Artificial cassette (PcURA3)
tgagaaacgtggcaatggatcattgtttatagaaaaatttaatgaatacgacaataatattaaaacaatttaatactgaaataaaagttgtaatatagtataaaatataaaattcatgagaaatatgtacaaaaggtttgtaagatcaccacattttctttaaaatgatctcaccataataataaaacatctaaagataaatcaaagggaacccacaaattgaaatgaaaagaattgtataaacatcatgactttaaacaattcacttctagtatatgagagataataaattcattaacagtattttttttttctaaattttttaattttttgtatctaaattctttaagcaaacaagaataaaagattaatacacctattaaatatctgaaccttaacgtctcatttgttgagttaataaagcattttgttcttggaatctttgaccgactctttcactgtgtttcaagaatttttcagaacattttaaaacacatgtattttcttttgaagttaatgaagcggaagtgaaatcattaacacaatcattgaaacaacgttcaaccaagtttgagtaaagacgcatgaaatctttcatttgtttaccttcaacgattctttggaaatcttgttgttctctttggtttaattgatccattttgattgatttgatatagatttgagctttgtagttctgatcaattaggtacaaaaggtctttcaatggcaaaagtgtacttttttgatttttcaatgaagtcgaaaaggttcaaatttttttttggtcaacaaaacatcataaatatccgaatttggaaagattcccgatatggacaaaatcaggaatcaattggaattatgattcatttgagcattatagtgtgaataattctttatgttctctgttctttattatatcaagctttaaagagacactaggcgtcccatagatcggatggtctattcaagtgtctcaaagaaaaaaaatagttgcttgattttggctgtagtagagcttgtacgggacacgcttctatgaataaatttgtccgatgagttggataaatattaactgaactaatttcttctaattgatagagcatcatcaatatattgcacataatataattcaaaaaaacaacaaacaacaacaactttacccagtggtacctacatacaattgacccatagtaaactaataactcataacacaataaagcatctgatcttaatgtactactaaatactaaactgatgataattacttttgttgtaatgtttgtcatcactttgatcatcacgagcatcaccggaccgttaattaccaacaatctcaattgtacaacatagtgttaaaacaggataacttgatgattatatgtgatattaagttcaaacaagtaccaataaatagataattaatagctctataatatatcatttaattgaattaatatcaatagttgttgtttaattatccctagttttctggttaaagttacaccatcagatggttcaccaccaatgttgttcaaaccatttccactcaactgacgtttccagaacatcaccctgaaaaaaaaaaattcatcacacattgggagaaattggggaggattgtatataaggagtggaaattcgctaatatttttataattctaactcacttgttttaattcaacatcagtattttataatacaaaaacaaacaaacaaacaaataattaattaacaatgggtactactttagatgatactgcttatagatatagaacttcagttccaggtgatgctgaagctattgaagctttagatggttcatttactactgatactgtttttagagttactgctactggtgatggttttactttaagagaagttccagttgatccaccattaactaaagtttttccagatgatgaatcagatgacgagtctgatgacggtgaagatggtgatccagattcaagaacttttgttgcttatggtgatgacggagacttagctggttttgttgttgtttcatattcaggttggaatagaagattaactgttgaagatattgaagttgctccagaacatagaggtcatggtgttggtagagctttaatgggtttagctactgaatttgctagagaacgtggtgctggtcatttatggttagaagttactaatgttaatgctccagctattcatgcttatagaagaatgggtttcacattatgtggtttagatactgctttatatgatggtactgcttcagatggtgaacaagctttatatatgtcaatgccatgtccataataagttgactgatttataattttattattattatttcaattcttattttttatcattaggtattaatgtggattatgttttaacttgttaatatataaattcacataaactaataattgtagatttttcgttatcattgaaaagcgtatactattaattatgaccccaggtgttggtcttgatgataaaggtgatgccttaggtcaacaatatagatccgttgataccgttgtttcaactggtagtgatatcattattgttggtagaggtttgttcggtaaaggaagagatccaaatgctgaaggtgaacgttacagagctgctggttggaatgcctatttgaaaagaactggtcaaatatagtatgtagtttaaatctaacatattagactaaataattaatgggtcataatttgtaattagttcaacgactaactaactgacattagaaggaagactctaattgtataccatgtcatcaatactcctaattatcaaataaatcaaaatatataccttctatcattaattagaagatgtaatgtcgatgactaagcaagataaattaaaaccgaaatccatctgtatgtaaaaatactttcaagtaattaccacatagatagaagctcaccaaccaactatcatcaagccagtagatgccattcaagagtgacaa

SEQ ID NO: 5 - DNA, 2289 bp, Artificial Sequence
  Artificial cassette (PcPOX3 cassette 1)
agtatcaaatcaattacttatacacttatgacttttatgacttttaaacgggtgatttctcttggactttcgaggaacatgctctaaatcaagcagagatcacaaatattttaataactaatgaataattttaaaattaaaggacttgtagcatattttgtggaatttccccatagtttattaatgtttttggaacctcggctttaatgggccctgcacaaatccgacggtccccaattgcacaaatccgacggcagccaatttgtttataaaagaaaaggaaaatcctttaatttcaaatccaaaacatcaacaaaaaagttggatctcaattggaaataggctgggaatcactgggaaatgagtgcacaggagtcagataggttgatccaggaaagggccattgagagggctggaacctcttttaacgtccaggatttgattcattatttagatgatggagaggaaaatactaaaatttatgaatcaatgtcacttcaattagaaagagatccaatttttaaaattaaatcttcacatttagatttaaaagccaaaagagaattagctttcaaaaaaattgtgaaattagctggttatggtcaacaatatagatccgttgataccgttgtttcaactggtagtgatatcattattgttggtagaggtttgttcggtaaaggaagagatccaaatgctgaaggtgaacgttacagagctgctggttggaatgcctatttgaaaagaactggtcaaatatagtatgtagtttaaatctaacatattagactaaataattaatgggtcataatttgtaattagttcaacgactaactaactgacattagaaggaagactctaattgtataccatgtcatcaatactcctaattatcaaataaatcaaaatatataccttctatcattaattagaagatgtaatgtcgatgactaagcaagataaattaaaaccgaaatccatctgtatgtaaaaatactttcaagtaattaccacatagatagaagctcaccaaccaactatcatcaagccagtagatgccattcaagagtgacaaatgtcattggaaaatgagttcacaggatcctcctttgagaatgagtttgaaaatactactgcccaaccagaattctgcagaattaattcgccctttttttttggtcaacaaaacatcataaatatccgaatttggaaagattcccgatatggacaaaatcaggaatcaattggaattatgattcatttgagcattatagtgtgaataattctttatgttctctgttctttattatatcaagctttaaagagacactaggcgtcccatagatcggatggtctattcaagtgtctcaaagaaaaaaaatagttgcttgattttggctgtagtagagcttgtacgggacacgcttctatgaataaatttgtccgatgagttggataaatattaactgaactaatttcttctaattgatagagcatcatcaatatattgcacataatataattcaaaatggttaccacattatcttattctcaaagagcagaagctcacccttctccattggcaaagcgtttattcaatgttatggaatcaaaaaagtcaaacttgtgtgcttcaattgatgttagaactacaaaagaatttttacaattagttgacacattaggtccatatatctgtcttgtcaaaactcatatcgatattattgatgatttctcattcgaaggtaccattaaaccattgaaagaattagcacaaaagcacaattttttaatctttgaagatcgtaaatttgctgatatagggaacacagtcaaagcacaatatgcaggtggtgctttcaaaattgcaacttggtctgatatcacaaatgctcatggtgttactggtgctggtatcgttagtggattgaaagaagctgctaaagaagcttctgatgaaccaagagggttgttgatgttggctgaattgagttcaaaaggttcattagccaaaggtgaatatactaaacaaactgttgatatcgctaaaactgataaagatttcgttattggttttattgctcaaaatgatatgggtggtagagatggaggctttgattggttaattatgaccccaggtgttggtcttgatgataaaggtgatgccttaggtcaacaatatagatccgttgataccgttgtttcaactggtagtgatatcattattgttggtagaggtttgttcggtaaaggaagagatccaaatgctgaaggtgaacgttacagagc

SEQ ID NO: 6 - DNA, 1671 bp, Artificial Sequence
  Artificial cassette (PcPOX3 cassette 2)
tttccattacatcagaaaacatttcacaattttattcattcaatatagttaaaggttcagattttttggaaaatttaaattataaaattgatgaaattaatgaattattaagacctgatattattggattaactgatgctttcaatttatcagattttgtaattgattctcaaattgggaaaagaaatggtgatatttatgaatcttatttcaaacatgttaatgataataattctgatttgaaacctcattattatgattctatcatgaaaccttttttccaaagagatatgaaacctagtgataatgaagaagttgatgaggaggaggaagaatagctacacacaccaacctctcaacaacttattatacattcttcttgacttttctatgacttttatagctttaaataaattcaaatttgatactttatactgattacgtaatacaaattcccccggtaaacacacacttttttttgtttacttttcaaaacatcaacaaaaaatttaaaacactttgaacgccaaaaaagaaggaaaaggaaaaccatcaaaaagatcgattgaagaagaagttagaaggatattaaggaaatatattaggtccatatatctgtcttgtcaaaactcatatcgatattattgatgatttctcattcgaaggtaccattaaaccattgaaagaattagcacaaaagcacaattttttaatctttgaagatcgtaaatttgctgatatagggaacacagtcaaagcacaatatgcaggtggtgctttcaaaattgcaacttggtctgatatcacaaatgctcatggtgttactggtgctggtatcgttagtggattgaaagaagctgctaaagaagcttctgatgaaccaagagggttgttgatgttggctgaattgagttcaaaaggttcattagccaaaggtgaatatactaaacaaactgttgatatcgctaaaactgataaagatttcgttattggttttattgctcaaaatgatatgggtggtagagatggaggctttgattggttaattatgaccccaggtgttggtcttgatgataaaggtgatgccttaggtcaacaatatagatccgttgataccgttgtttcaactggtagtgatatcattattgttggtagaggtttgttcggtaaaggaagagatccaaatgctgaaggtgaacgttacagagctgctggttggaatgcctatttgaaaagaactggtcaaatatagtatgtagtttaaatctaacatattagactaaataattaatgggtcataatttgtaattagttcaacgactaactaactgacattagaaggaagactctaattgtataccatgtcatcaatactcctaattatcaaataaatcaaaatatataccttctatcattaattagaagatgtaatgtcgatgactaagcaagataaattaaaaccgaaatccatctgtatgtaaaaatactttcaagtaattaccacatagatagaagctcaccaaccaactatcatcaagccagtagatgccattcaagagtgacaaatgtcattggaaaatgagttcacaggatcctcctttgagaatgagtttgaaaatactactgcccaaccagaattaagggcgaattccagcacactggcggccgtta

SEQ ID NO: 7 - DNA, 2799 bp, Artificial Sequence
  Artificial cassette (PcLCB4 cassette 1)
aaacttattctcttgtttggaacacattacaacacattttagttaaagtcttgttggcgaaactggtatcaagaaaacgtttcacaactttatcattttgatataaagacatacttcaacccatccatacacttatttgaactcttttttgcccttttcatcatgccgagttttgactctcaaagaattaaactgatggatacagtatcagtaaacccccaagagccatcattggtgatacaggtatcatcattaaagatcaatcttcattctattacaatcaacatgataacgcttcattttcatcttgcttaagttgctcttcatcaaactcgaatggtacggtgaaatcttcaggtccaaaacatattccatttgttgatatattgagtgttcgatatataaatgaaaataatgaatctttattagaagctggaagttccactgtgactagtgatgaacctgatgtcgaagtggtatttgttagacaaaagggtaaaactcttgtaccaactccaataatattatcaatagatactttaggtcatgatgatgttgtacaagaaatttggagattaagttatcaaggaacaaaccaagaaaatcaatattagttcttgttaatccacatggtgggaaaggtaaagctataaattcattctaactcaatcaaaacctgtattaattggtgctcaagcttctgttgaagttagacatactcaatattatcaacatgctacagatattgcacgcactttgaatattgataaatatgatataattgcatgtgcttcaggtgatggtgtcccacatgaagtcttgaatggattttatcaaagatctgatagagctgaagctttcaataagattacaataactcaattaccatgtggttcaggtaatgcaatgagtgaatcatgtcatggtacaaataatccaagttttgccgctctatcattattgaaatcaagtacggtaaatttagatttaatggcttgtacacaaggtgataaaacttatgtttcattcttaagtcaaactgtcggtgttatagcagattctgatattggtactgaagcacttagatggttaggtccttcaagatttgaaggtcaacaatatagatccgttgataccgttgtttcaactggtagtgatatcattattgttggtagaggtttgttcggtaaaggaagagatccaaatgctgaaggtgaacgttacagagctgctggttggaatgcctatttgaaaagaactggtcaaatatagtatgtagtttaaatctaacatattagactaaataattaatgggtcataatttgtaattagttcaacgactaactaactgacattagaaggaagactctaattgtataccatgtcatcaatactcctaattatcaaataaatcaaaatatataccttctatcattaattagaagatgtaatgtcgatgactaagcaagataaattaaaaccgaaatccatctgtatgtaaaaatactttcaagtaattaccacatagatagaagctcaccaaccaactatcatcaagccagtagatgccattcaagagtgacaaatgtcattggaaaatgagttcacaggatcctcctttgagaatgagtttgaaaatactactgcccaaccagaattctgcagaattaattcgccctttttttttggtcaacaaaacatcataaatatccgaatttggaaagattcccgatatggacaaaatcaggaatcaattggaattatgattcatttgagcattatagtgtgaataattctttatgttctctgttctttattatatcaagctttaaagagacactaggcgtcccatagatcggatggtctattcaagtgtctcaaagaaaaaaaatagttgcttgattttggctgtagtagagcttgtacgggacacgcttctatgaataaatttgtccgatgagttggataaatattaactgaactaatttcttctaattgatagagcatcatcaatatattgcacataatataattcaaaatggttaccacattatcttattctcaaagagcagaagctcacccttctccattggcaaagcgtttattcaatgttatggaatcaaaaaagtcaaacttgtgtgcttcaattgatgttagaactacaaaagaatttttacaattagttgacacattaggtccatatatctgtcttgtcaaaactcatatcgatattattgatgatttctcattcgaaggtaccattaaaccattgaaagaattagcacaaaagcacaattttttaatctttgaagatcgtaaatttgctgatatagggaacacagtcaaagcacaatatgcaggtggtgctttcaaaattgcaacttggtctgatatcacaaatgctcatggtgttactggtgctggtatcgttagtggattgaaagaagctgctaaagaagcttctgatgaaccaagagggttgttgatgttggctgaattgagttcaaaaggttcattagccaaaggtgaatatactaaacaaactgttgatatcgctaaaactgataaagatttcgttattggttttattgctcaaaatgatatgggtggtagagatggaggctttgattggttaattatgaccccaggtgttggtcttgatgataaaggtgatgccttaggtcaacaatatagatccgttgataccgttgtttcaactggtagtgatatcattattgttggtagaggtttgttcggtaaaggaagagatccaaatgctgaaggtgaacgttacagagc

SEQ ID NO: 8 - DNA, 2278 bp, Artificial Sequence
  Artificial cassette (PcLCB4 cassette 2)
cgtatggcaccaactttattatcattagatcaaggttctcatgttttacaaccagaagttcaacattctaaaataatagcatatagattaactccaaagcagcaacatggttatttaagtgttgatggtgaaagttatccatttgaaactattcaagttgaaattctacccggtgctgcaaagactttactaagaaatggtacttatgttgaaacaaatttttattgaaatgaatgataaattttgatgcttacatatatatatatattatctctaacgaatgaaacgaatatgatacttacaatctgattacacaaatatttaattgtagtcaacttataattgttgaatttaaaatttgatttaatttttgaagctttaatggagatgccgatgttggataaaccgggttttgaaaatctttttgactccatactaaaaaattaagtgctgatgagtaacttaaggaacgtcaagtcatagaagtaattgttttatttcaaatttttataaattaagcgctttttccttcagttgttttttttttgttggtttatttattactcaaaaatttctaaataataacataaattatagaaatcatgagtgaagacgaacaagaatttgctaaattagaacaaactttaccagactcaatcaagagttcatcatcacatattttcaatcaagaatttttaaattcaattaatcatactccatcattaactccacaaagttcaataccgccagaatcaccaaaattgccaaagaaaactccattaagtaattttaaagatgaattatataaaaatggtgatgtcgaaagaacccattcaccaattccaacaccaggtcctttacttcatcctgatgttcatttcccagctttgaataagcaaaatgcagctactggtgttatttggtgtactgatcgtgcaaatgaacgtggtttcccaaatccaaattgggtcaatttaggtcaaggtatgccagaaacaggtgatattccaggatgttttgataggccaaaatcaatgaatatttcaattgaatctcgtgaatatggtccaacatctggtattaaacctttaagacaagctattgcaaatttatataatgaacattatagacaaggtaaagaatcaaaatatacttgggaaaatgtcaatgttgcaccaggtggcagagctgctttaacaagaattgcattaggtccatatatctgtcttgtcaaaactcatatcgatattattgatgatttctcattcgaaggtaccattaaaccattgaaagaattagcacaaaagcacaattttttaatctttgaagatcgtaaatttgctgatatagggaacacagtcaaagcacaatatgcaggtggtgctttcaaaattgcaacttggtctgatatcacaaatgctcatggtgttactggtgctggtatcgttagtggattgaaagaagctgctaaagaagcttctgatgaaccaagagggttgttgatgttggctgaattgagttcaaaaggttcattagccaaaggtgaatatactaaacaaactgttgatatcgctaaaactgataaagatttcgttattggttttattgctcaaaatgatatgggtggtagagatggaggctttgattggttaattatgaccccaggtgttggtcttgatgataaaggtgatgccttaggtcaacaatatagatccgttgataccgttgtttcaactggtagtgatatcattattgttggtagaggtttgttcggtaaaggaagagatccaaatgctgaaggtgaacgttacagagctgctggttggaatgcctatttgaaaagaactggtcaaatatagtatgtagtttaaatctaacatattagactaaataattaatgggtcataatttgtaattagttcaacgactaactaactgacattagaaggaagactctaattgtataccatgtcatcaatactcctaattatcaaataaatcaaaatatataccttctatcattaattagaagatgtaatgtcgatgactaagcaagataaattaaaaccgaaatccatctgtatgtaaaaatactttcaagtaattaccacatagatagaagctcaccaaccaactatcatcaagccagtagatgccattcaagagtgacaaatgtcattggaaaatgagttcacaggatcctcctttgagaatgagtttgaaaatactactgcccaaccagaattaagggcgaattccagcacactggcggccgtta

SEQ ID NO: 9 - DNA, 23 bp, Artificial Sequence
  nat1_MB primer
ttcaacggttaatctacggttcc

SEQ ID NO: 10 - DNA, 25 bp, Artificial Sequence
  PcURA3_5D1F primer
tgagaaacgtggcaatggatcattg

SEQ ID NO: 11 - DNA, 21 bp, Artificial Sequence
  nat1_1F primer
atgaccactttggatgacacc

SEQ ID NO: 12 - DNA, 26 bp, Artificial Sequence
  PcURA3_3D2B primer
ttgtcactcttgaatggcatctactg

SEQ ID NO: 13 - DNA, 20 bp, Artificial Sequence
  PCura3R primer
gctctgtaacgttcaccttc

SEQ ID NO: 14 - DNA, 25 bp, Artificial Sequence
  PCura3F primer
attaggtccatatatctgtcttgtc

SEQ ID NO: 15 - DNA, 54 bp, Artificial Sequence
  PcPOX3 N1
gatgcatgctcgagcagtatcaaatcaattacttatacacttatgacttttatg

SEQ ID NO: 16 - DNA, 39 bp, Artificial Sequence
  PcPOX3 N2
agtatcaaatcaattacttatacacttatgacttttatg

SEQ ID NO: 17 - DNA, 49 bp, Artificial Sequence
  PcPOX3 N3
tatattgttgaccgcataaccagctaatttcacaatttttttgaaagct

SEQ ID NO: 18 - DNA, 45 bp, Artificial Sequence
  PcPOX3 N4
cactggcggccgttatttccattacatcagaaaacatttcacaat

SEQ ID NO: 19 - DNA, 49 bp, Artificial Sequence
  PcPOX3 N5
ccgagctcggatccaatatttccttaatatccttctaacttcttcttca

SEQ ID NO: 20 - DNA, 34 bp, Artificial Sequence
  PcPOX3 N6
atatttccttaatatccttctaacttcttcttca

SEQ ID NO: 21 - DNA, 40 bp, Artificial Sequence
  PcLCB4 N1
gatgcatgctcgagcaaacttattctcttgtttggaacac

SEQ ID NO: 22 - DNA, 25 bp, Artificial Sequence
  PcLCB4 N2
aaacttattctcttgtttggaacac

SEQ ID NO: 23 - DNA, 38 bp, Artificial Sequence
  PcLCB4 N3
tatattgttgaccgcttcaaatcttgaaggacctaacc

SEQ ID NO: 24 - DNA, 38 bp, Artificial Sequence
  PcLCB4 N4
cactggcggccgttacgtatggcaccaactttattatc

SEQ ID NO: 25 - DNA, 37 bp, Artificial Sequence
  PcLCB4 N5
ccgagctcggatccagcaattcttgttaaagcagctc

SEQ ID NO: 26 - DNA, 22 bp, Artificial Sequence
  PcLCB4 N6
gcaattcttgttaaagcagctc

SEQ ID NO: 27 - DNA, 150 bp, Pichia ciferrii
  gene (1)..(150): T-TEF
gttgactgatttataattttattattattatttcaattcttattttttatcattaggtattaatgtggattatgttttaacttgttaatatataaattcacataaactaataattgtagatttttcgttatcattgaaaagcgtatacta

SEQ ID NO: 28 - DNA, 2049 bp, Pichia ciferrii
  gene (1)..(2049): POX3 gene
atgagtgcacaggagtcagataggttgatccaggaaagggccattgagagggctggaacctcttttaacgtccaggatttgattcattatttagatgatggagaggaaaatactaaaatttatgaatcaatgtcacttcaattagaaagagatccaatttttaaaattaaatcttcacatttagatttaaaagccaaaagagaattagctttcaaaaaaattgtgaaattagctggttatttccaaaactctgatgaagttgaactacgtaatagaattagaattctttcacttattgatccggatgttgctacaagaattggtgttcattatgggttattcattggtactctaagagctcttggttcttcaaaacaatttgaattttggatcaagaaaggtgctttttcattatcaaatttttatggatgttttgcaatgactgaattagctcatggttctaatgttgcagctttacaaacaactgcaacttatgatccacaagatgaaacttttatcatccatacaccttcattaagtgctacaaaatggtggattggtggcgctgctcattcagctactcatgctgttgtttatgctagattaatctcccagggaaaggattatggtgttaagaatttcattgttcaattaagaaattctcaacatgaattattaccaggtgtttcagttggtgatattggtaaaaaaatgggtagagatggtattgataatggttggattcaattcacaaatgttaaaatccctaaattcaatatgttggataaatatgctaaagttgataatgatggtaaagttacattacctcaattccaacaattaggttatactgcattagttgttggtagagtctcaatggttgttgattcttataacactggtaagaaatttttaacaattgcattaagatatgcatcaacaagaagacaatttggtaaagattctgaagggaaagagaaaaaaatcattgattatacacatcatagaagaagattattcccattattagctagtgtttatgcaatgaattcagctgctttagttatttcaaaatttcaagatgaagctaataaacttgttgaaagtggtgaaaatttaaaacatgtgattccaaatttaaaagatctttttggtctttcagctggattaaaggcattttgtacttgggaaactgctcatattattgatgaaacaagacaaagttgtggtggtcatggttattcagattataatgcttttgcaagaggttataatgattgggttgttcaatgtacttgggaaggtgataataatgttttatcaatgagttgtggtagagctttaattcaaaattatctaagtgttgaaaagaagaaaattgtggggaaatatacaaaatatttagaaaccacagatatttcaaatgaatttgaattaaaatctcaagatttagaatatattgaaaaaataattaaagcttgggaatttgtttctaagagtttaattgttaaatcaacaaataaatttaaaaattttgttaaagaatttaatggtgatgttgaattagcatttgaaaaaatctcatcatatagatttattattgctaaagttcatacaaaattaatccttttgaaatcattttatgaaagaattttggaagcaccaaagaatttaaaaccagttctgtcattattattacaattatattctctttccattacatcagaaaacatttcacaattttattcattcaatatagttaaaggttcagattttttggaaaatttaaattataaaattgatgaaattaatgaattattaagacctgatattattggattaactgatgctttcaatttatcagattttgtaattgattctcaaattgggaaaagaaatggtgatatttatgaatcttatttcaaacatgttaatgataataattctgatttgaaacctcattattatgattctatcatgaaaccttttttccaaagagatatgaaacctagtgataatgaagaagttgatgaggaggaggaagaatag

SEQ ID NO: 29 - DNA, 1530 bp, Pichia ciferrii
  gene (1)..(1530): LCB4 gene
atgccgagttttgactctcaaagaattaaactgatggatacagtatcagtaaaccccccaagagccatcattggtgatacaggtatcatcattaaagatcaatcttcattctattacaatcaacatgataacgcttcattttcatcttgcttaagttgctcttcatcaaactcgaatggtacggtgaaatcttcaggtccaaaacatattccatttgttgatatattgagtgttcgatatataaatgaaaataatgaatctttattagaagctggaagttccactgtgactagtgatgaacctgatgtcgaagtggtatttgttagacaaaagggtaaaactcttgtaccaactccaataatattatcaatagatactttaggtcatgatgatgttgtacaagaaatttggagattaagttatcaaggaacaaaaccaagaaaatcaatattagttcttgttaatccacatggtgggaaaggtaaagctataaattcattcttaactcaatcaaaacctgtattaattggtgctcaagcttctgttgaagttagacatactcaatattatcaacatgctacagatattgcacgcactttgaatattgataaatatgatataattgcatgtgcttcaggtgatggtgtcccacatgaagtcttgaatggattttatcaaagatctgatagagctgaagctttcaataagattacaataactcaattaccatgtggttcaggtaatgcaatgagtgaatcatgtcatggtacaaataatccaagttttgccgctctatcattattgaaatcaagtacggtaaatttagatttaatggcttgtacacaaggtgataaaacttatgtttcattcttaagtcaaactgtcggtgttatagcagattctgatattggtactgaagcacttagatggttaggtccttcaagatttgaattaggtgttgcttataaagttttatcaagatcaagatatccatgtgatatatctgttaaatatgctgcaaaatcgaaaaatgaattaagacaacattttgatgaacattccactattgtttcaacaaaagatatccaaataactgaagatacttataatttaaaatatgatccaaatggtccaatacctgatgattgggaagagattgataaagatctttcagaaaatttaggtattttctatacaggtaaaatgccatatattgcaaaagatgttcaatttttccctgcagctttaccaaatgatggtacttttgatttagttataacagatgctcgtacaagtatagcacgtatggcaccaactttattatcattagatcaaggttctcatgttttacaaccagaagttcaacattctaaaataatagcatatagattaactccaaagcagcaacatggttatttaagtgttgatggtgaaagttatccatttgaaactattcaagttgaaattctacccggtgctgcaaagactttactaagaaatggtacttatgttgaaacaaatttttattga